European Patent Application EP 4 516 913 A1, published March 5, 2025. Title: AAV vector introduced with hepatocyte growth factor gene optimized for intrathecal administration. Applicant: Helixmith Co., Ltd. The sequence listing filed with the application follows.

SEQUENCE LISTING (20 sequences)

SEQ ID NO: 1 - protein, 728 aa, synthetic construct
  REGION 1..728: note = Full-length HGF
MWVTKLLPALLLQHVLLHLLLLPIAIPYAEGQRKRRNTIHEFKKSAKTTLIKIDPALKIKTKKVNTADQCANRCTRNKGLPFTCKAFVFDKARKQCLWFPFNSMSSGVKKEFGHEFDLYENKDYIRNCIIGKGRSYKGTVSITKSGIKCQPWSSMIPHEHSFLPSSYRGKDLQENYCRNPRGEEGGPWCFTSNPEVRYEVCDIPQCSEVECMTCNGESYRGLMDHTESGKICQRWDHQTPHRHKFLPERYPDKGFDDNYCRNPDGQPRPWCYTLDPHTRWEYCAIKTCADNTMNDTDVPLETTECIQGQGEGYRGTVNTIWNGIPCQRWDSQYPHEHDMTPENFKCKDLRENYCRNPDGSESPWCFTTDPNIRVGYCSQIPNCDMSHGQDCYRGNGKNYMGNLSQTRSGLTCSMWDKNMEDLHRHIFWEPDASKLNENYCRNPDDDAHGPWCYTGNPLIPWDYCPISRCEGDTTPTIVNLDHPVISCAKTKQLRVVNGIPTRTNIGWMVSLRYRNKHICGGSLIKESWVLTARQCFPSRDLKDYEAWLGIHDVHGRGDEKCKQVLNVSQLVYGPEGSDLVLMKLARPAVLDDFVSTIDLPNYGCTIPEKTSCSVYGWGYTGLINYDGLLRVAHLYIMGNEKCSQHHRGKVTLNESEICAGAEKIGSGPCEGDYGGPLVCEQHKMRMVLGVIVPGRGCAIPNRPGIFVRVAYYAKWIHKIILTYKVPQS

SEQ ID NO: 2 - protein, 723 aa, synthetic construct
  REGION 1..723: note = Deleted variant HGF
MWVTKLLPALLLQHVLLHLLLLPIAIPYAEGQRKRRNTIHEFKKSAKTTLIKIDPALKIKTKKVNTADQCANRCTRNKGLPFTCKAFVFDKARKQCLWFPFNSMSSGVKKEFGHEFDLYENKDYIRNCIIGKGRSYKGTVSITKSGIKCQPWSSMIPHEHSYRGKDLQENYCRNPRGEEGGPWCFTSNPEVRYEVCDIPQCSEVECMTCNGESYRGLMDHTESGKICQRWDHQTPHRHKFLPERYPDKGFDDNYCRNPDGQPRPWCYTLDPHTRWEYCAIKTCADNTMNDTDVPLETTECIQGQGEGYRGTVNTIWNGIPCQRWDSQYPHEHDMTPENFKCKDLRENYCRNPDGSESPWCFTTDPNIRVGYCSQIPNCDMSHGQDCYRGNGKNYMGNLSQTRSGLTCSMWDKNMEDLHRHIFWEPDASKLNENYCRNPDDDAHGPWCYTGNPLIPWDYCPISRCEGDTTPTIVNLDHPVISCAKTKQLRVVNGIPTRTNIGWMVSLRYRNKHICGGSLIKESWVLTARQCFPSRDLKDYEAWLGIHDVHGRGDEKCKQVLNVSQLVYGPEGSDLVLMKLARPAVLDDFVSTIDLPNYGCTIPEKTSCSVYGWGYTGLINYDGLLRVAHLYIMGNEKCSQHHRGKVTLNESEICAGAEKIGSGPCEGDYGGPLVCEQHKMRMVLGVIVPGRGCAIPNRPGIFVRVAYYAKWIHKIILTYKVPQS

SEQ ID NO: 3 - DNA, 7377 bp, synthetic construct
  misc_feature 1..7377: note = Hybrid HGF
  source 1..7377: mol_type = other DNA
cgcgttgacattgattattgactagttattaatagtaatcaattacggggtcattagttcatagcccatatatggagttccgcgttacataacttacggtaaatggcccgcctggctgaccgcccaacgacccccgcccattgacgtcaataatgacgtatgttcccatagtaacgccaatagggactttccattgacgtcaatgggtggagtatttacggtaaactgcccacttggcagtacatcaagtgtatcatatgccaagtccgccccctattgacgtcaatgacggtaaatggcccgcctggcattatgcccagtacatgaccttacgggactttcctacttggcagtacatctacgtattagtcatcgctattaccatggtgatgcggttttggcagtacaccaatgggcgtggatagcggtttgactcacggggatttccaagtctccaccccattgacgtcaatgggagtttgttttggcaccaaaatcaacgggactttccaaaatgtcgtaataaccccgccccgttgacgcaaatgggcggtaggcgtgtacggtgggaggtctatataagcagagctcgtttagtgaaccgtcagatcgcctggagacgccatccacgctgttttgacctccatagaagacaccgggaccgatccagcctccgcggccgggaacggtgcattggaacgcggattccccgtgccaagagtgacgtaagtaccgcctatagactctataggcacacccctttggctcttatgcatgctatactgtttttggcttggggcctatacacccccgcttccttatgctataggtgatggtatagcttagcctataggtgtgggttattgaccattattgaccactcccctattggtgacgatactttccattactaatccataacatggctctttgccacaactatctctattggctatatgccaatactctgtccttcagagactgacacggactctgtatttttacaggatggggtcccatttattatttacaaattcacatatacaacaacgccgtcccccgtgcccgcagtttttattaaacatagcgtgggatctccacgcgaatctcgggtacgtgttccggacatgggctcttctccggtagcggcggagcttccacatccgagccctggtcccatgcctccagcggctcatggtcgctcggcagctccttgctcctaacagtggaggccagacttaggcacagcacaatgcccaccaccaccagtgtgccgcacaaggccgtggcggtagggtatgtgtctgaaaatgagctcggagattgggctcgcaccgctgacgcagatggaagacttaaggcagcggcagaagaagatgcaggcagctgagttgttgtattctgataagagtcagaggtaactcccgttgcggtgctgttaacggtggagggcagtgtagtctgagcagtactcgttgctgccgcgcgcgccaccagacataatagctgacagactaacagactgttcctttccatgggtcttttctgcagtcaccgtccttgacacgaagcttgctagcaccatgtgggtgaccaaactcctgccagccctgctgctgcagcatgtcctcctgcatctcctcctgctccccatcgccatcccctatgcagagggacaaaggaaaagaagaaatacaattcatgaattcaaaaaatcagcaaagactaccctaatcaaaatagatccagcactgaagataaaaaccaaaaaagtgaatactgcagaccaatgtgctaatagatgtactaggaataaaggacttccattcacttgcaaggcttttgtttttgataaagcaagaaaacaatgcctctggttccccttcaatagcatgtcaagtggagtgaaaaaagaatttggccatgaatttgacctctatgaaaacaaagactacattagaaactgcatcattggtaaaggacgcagctacaagggaacagtatctatcactaagagtggcatcaaatgtcagccctggagttccatgataccacacgaacacaggtaagaacagtatgaagaaaagagatgaagcctctgtcttttttacatgttaacagtctcatattagtccttcagaataattctacaatcctaaaataacttagccaacttgctgaattgtattacggcaaggtttatatgaattcatgactgatatttagcaaatgattaattaatatgttaataaaatgtagccaaaacaatatcttaccttaatgcctcaatttgtagatctcggtatttgtggatcctgggtaggaaacacatttgaatggtatttactaagatactaaaatccttggacttcactctaattttagtgccatttagaactcaaggtctcagtaaaagtagaaataaagcctgttaacaaaacacaaactgaatattaaaaatgtaactggattttcaaagaaatgtttactggtattacctgtagatgtatattctttattatgatcttttgtgtaaagtctggcagacaaatgcaatatctaattgttgagtccaatatcacaagcagtacaaaagtataaaaaagacttggccttttctaatgtgttaaaatactttatgctggtaataacactaagagtagggcactagaaattttaagtgaagataatgtgttgcagttactgcactcaatggcttactattataaaccaaaactgggatcactaagctccagtcagtcaaaatgatcaaaattattgaagagaataagcaattctgttctttattaggacacagtagatacagactacaaagtggagtgtgcttaataagaggtagcatttgttaagtgtcaattactctattatcccttggagcttctcaaaataaccatataaggtgtaagatgttaaaggttatggttacactcagtgcacaggtaagctaataggctgagagaagctaaattacttactggggtctcacagtaagaaagtgagctgaagtttcagcccagatttaactggattctgggctctttattcatgttacttcatgaatctgtttctcaattgtgcagaaaaaagggggctatttataagaaaagcaataaacaaacaagtaatgatctcaaataagtaatgcaagaaatagtgagatttcaaaatcagtggcagcgatttctcagttctgtcctaagtggccttgctcaatcacctgctatcttttagtggagctttgaaattatgtttcagacaacttcgattcagttctagaatgtttgactcagcaaattcacaggctcatctttctaacttgatggtgaatatggaaattcagctaaatggatgttaataaaattcaaacgttttaaggacagatggaaatgacagaattttaaggtaaaatatatgaaggaatataagataaaggatttttctaccttcagcaaaaacatacccactaattagtaaaattaataggcgaaaaaaagttgcatgctcttatactgtaatgattatcattttaaaactagctttttgccttcgagctatcggggtaaagacctacaggaaaactactgtcgaaatcctcgaggggaagaagggggaccctggtgtttcacaagcaatccagaggtacgctacgaagtctgtgacattcctcagtgttcagaagttgaatgcatgacctgcaatggggagagttatcgaggtctcatggatcatacagaatcaggcaagatttgtcagcgctgggatcatcagacaccacaccggcacaaattcttgcctgaaagatatcccgacaagggctttgatgataattattgccgcaatcccgatggccagccgaggccatggtgctatactcttgaccctcacacccgctgggagtactgtgcaattaaaacatgcgctgacaatactatgaatgacactgatgttcctttggaaacaactgaatgcatccaaggtcaaggagaaggctacaggggcactgtcaataccatttggaatggaattccatgtcagcgttgggattctcagtatcctcacgagcatgacatgactcctgaaaatttcaagtgcaaggacctacgagaaaattactgccgaaatccagatgggtctgaatcaccctggtgttttaccactgatccaaacatccgagttggctactgctcccaaattccaaactgtgatatgtcacatggacaagattgttatcgtgggaatggcaaaaattatatgggcaacttatcccaaacaagatctggactaacatgttcaatgtgggacaagaacatggaagacttacatcgtcatatcttctgggaaccagatgcaagtaagctgaatgagaattactgccgaaatccagatgatgatgctcatggaccctggtgctacacgggaaatccactcattccttgggattattgccctatttctcgttgtgaaggtgataccacacctacaatagtcaatttagaccatcccgtaatatcttgtgccaaaacgaaacaattgcgagttgtaaatgggattccaacacgaacaaacataggatggatggttagtttgagatacagaaataaacatatctgcggaggatcattgataaaggagagttgggttcttactgcacgacagtgtttcccttctcgagacttgaaagattatgaagcttggcttggaattcatgatgtccacggaagaggagatgagaaatgcaaacaggttctcaatgtttcccagctggtatatggccctgaaggatcagatctggttttaatgaagcttgccaggcctgctgtcctggatgattttgttagtacgattgatttacctaattatggatgcacaattcctgaaaagaccagttgcagtgtttatggctggggctacactggattgatcaactatgatggcctattacgagtggcacatctctatataatgggaaatgagaaatgcagccagcatcatcgagggaaggtgactctgaatgagtctgaaatatgtgctggggctgaaaagattggatcaggaccatgtgagggggattatggtggcccacttgtttgtgagcaacataaaatgagaatggttcttggtgtcattgttcctggtcgtggatgtgccattccaaatcgtcctggtatttttgtccgagtagcatattatgcaaaatggatacacaaaattattttaacatataaggtaccacagtcatagcggccgctctagagggcccgtttaaacccgctgatcagcctcgactgtgccttctagttgccagccatctgttgtttgcccctcccccgtgccttccttgaccctggaaggtgccactcccactgtcctttcctaataaaatgaggaaattgcatcgcattgtctgagtaggtgtcattctattctggggggtggggtggggcaggacagcaagggggaggattgggaagacaatagcaggcatgctggggagtcgaaattcagaagaactcgtcaagaaggcgatagaaggcgatgcgctgcgaatcgggagcggcgataccgtaaagcacgaggaagcggtcagcccattcgccgccaagctcttcagcaatatcacgggtagccaacgctatgtcctgatagcggtccgccacacccagccggccacagtcgatgaatccagaaaagcggccattttccaccatgatattcggcaagcaggcatcgccatgggtcacgacgagatcctcgccgtcgggcatgctcgccttgagcctggcgaacagttcggctggcgcgagcccctgatgctcttcgtccagatcatcctgatcgacaagaccggcttccatccgagtacgtgctcgctcgatgcgatgtttcgcttggtggtcgaatgggcaggtagccggatcaagcgtatgcagccgccgcattgcatcagccatgatggatactttctcggcaggagcaaggtgagatgacaggagatcctgccccggcacttcgcccaatagcagccagtcccttcccgcttcagtgacaacgtcgagcacagctgcgcaaggaacgcccgtcgtggccagccacgatagccgcgctgcctcgtcttgcagttcattcagggcaccggacaggtcggtcttgacaaaaagaaccgggcgcccctgcgctgacagccggaacacggcggcatcagagcagccgattgtctgttgtgcccagtcatagccgaatagcctctccacccaagcggccggagaacctgcgtgcaatccatcttgttcaatcatgcgaaacgatcctcatcctgtctcttgatcagatcttgatcccctgcgccatcagatccttggcggcaagaaagccatccagtttactttgcagggcttcccaaccttaccagagggcgccccagctggcaattccggttcgcttgctgtccataaaaccgcccagtctagctatcgccatgtaagcccactgcaagctacctgctttctctttgcgcttgcgttttcccttgtccagatagcccagtagctgacattcatccggggtcagcaccgtttctgcggactggctttctacgtgaaaaggatctaggtgaagatcctttttgataatctcatgaccaaaatcccttaacgtgagttttcgttccactgagcgtcagaccccgtagaaaagatcaaaggatcttcttgagatcctttttttctgcgcgtaatctgctgcttgcaaacaaaaaaaccaccgctaccagcggtggtttgtttgccggatcaagagctaccaactctttttccgaaggtaactggcttcagcagagcgcagataccaaatactgttcttctagtgtagccgtagttaggccaccacttcaagaactctgtagcaccgcctacatacctcgctctgctaatcctgttaccagtggctgctgccagtggcgataagtcgtgtcttaccgggttggactcaagacgatagttaccggataaggcgcagcggtcgggctgaacggggggttcgtgcacacagcccagcttggagcgaacgacctacaccgaactgagatacctacagcgtgagctatgagaaagcgccacgcttcccgaagggagaaaggcggacaggtatccggtaagcggcagggtcggaacaggagagcgcacgagggagcttccagggggaaacgcctggtatctttatagtcctgtcgggtttcgccacctctgacttgagcgtcgatttttgtgatgctcgtcaggggggcggagcctatggaaaaacgccagcaacgcggcctttttacggttcctggccttttgctggccttttgctcacatg

SEQ ID NO: 4 - DNA, 3679 bp, synthetic construct
  misc_feature 1..3679: note = HGF-X7
  source 1..3679: mol_type = other DNA
atgtgggtgaccaaactcctgccagccctgctgctgcagcatgtcctcctgcatctcctcctgctccccatcgccatcccctatgcagagggacaaaggaaaagaagaaatacaattcatgaattcaaaaaatcagcaaagactaccctaatcaaaatagatccagcactgaagataaaaaccaaaaaagtgaatactgcagaccaatgtgctaatagatgtactaggaataaaggacttccattcacttgcaaggcttttgtttttgataaagcaagaaaacaatgcctctggttccccttcaatagcatgtcaagtggagtgaaaaaagaatttggccatgaatttgacctctatgaaaacaaagactacattagaaactgcatcattggtaaaggacgcagctacaagggaacagtatctatcactaagagtggcatcaaatgtcagccctggagttccatgataccacacgaacacaggtaagaacagtatgaagaaaagagatgaagcctctgtcttttttacatgttaacagtctcatattagtccttcagaataattctacaatcctaaaataacttagccaacttgctgaattgtattacggcaaggtttatatgaattcatgactgatatttagcaaatgattaattaatatgttaataaaatgtagccaaaacaatatcttaccttaatgcctcaatttgtagatctcggtatttgtggatcctgggtaggaaacacatttgaatggtatttactaagatactaaaatccttggacttcactctaattttagtgccatttagaactcaaggtctcagtaaaagtagaaataaagcctgttaacaaaacacaaactgaatattaaaaatgtaactggattttcaaagaaatgtttactggtattacctgtagatgtatattctttattatgatcttttgtgtaaagtctggcagacaaatgcaatatctaattgttgagtccaatatcacaagcagtacaaaagtataaaaaagacttggccttttctaatgtgttaaaatactttatgctggtaataacactaagagtagggcactagaaattttaagtgaagataatgtgttgcagttactgcactcaatggcttactattataaaccaaaactgggatcactaagctccagtcagtcaaaatgatcaaaattattgaagagaataagcaattctgttctttattaggacacagtagatacagactacaaagtggagtgtgcttaataagaggtagcatttgttaagtgtcaattactctattatcccttggagcttctcaaaataaccatataaggtgtaagatgttaaaggttatggttacactcagtgcacaggtaagctaataggctgagagaagctaaattacttactggggtctcacagtaagaaagtgagctgaagtttcagcccagatttaactggattctgggctctttattcatgttacttcatgaatctgtttctcaattgtgcagaaaaaagggggctatttataagaaaagcaataaacaaacaagtaatgatctcaaataagtaatgcaagaaatagtgagatttcaaaatcagtggcagcgatttctcagttctgtcctaagtggccttgctcaatcacctgctatcttttagtggagctttgaaattatgtttcagacaacttcgattcagttctagaatgtttgactcagcaaattcacaggctcatctttctaacttgatggtgaatatggaaattcagctaaatggatgttaataaaattcaaacgttttaaggacagatggaaatgacagaattttaaggtaaaatatatgaaggaatataagataaaggatttttctaccttcagcaaaaacatacccactaattagtaaaattaataggcgaaaaaaagttgcatgctcttatactgtaatgattatcattttaaaactagctttttgccttcgagctatcggggtaaagacctacaggaaaactactgtcgaaatcctcgaggggaagaagggggaccctggtgtttcacaagcaatccagaggtacgctacgaagtctgtgacattcctcagtgttcagaagttgaatgcatgacctgcaatggggagagttatcgaggtctcatggatcatacagaatcaggcaagatttgtcagcgctgggatcatcagacaccacaccggcacaaattcttgcctgaaagatatcccgacaagggctttgatgataattattgccgcaatcccgatggccagccgaggccatggtgctatactcttgaccctcacacccgctgggagtactgtgcaattaaaacatgcgctgacaatactatgaatgacactgatgttcctttggaaacaactgaatgcatccaaggtcaaggagaaggctacaggggcactgtcaataccatttggaatggaattccatgtcagcgttgggattctcagtatcctcacgagcatgacatgactcctgaaaatttcaagtgcaaggacctacgagaaaattactgccgaaatccagatgggtctgaatcaccctggtgttttaccactgatccaaacatccgagttggctactgctcccaaattccaaactgtgatatgtcacatggacaagattgttatcgtgggaatggcaaaaattatatgggcaacttatcccaaacaagatctggactaacatgttcaatgtgggacaagaacatggaagacttacatcgtcatatcttctgggaaccagatgcaagtaagctgaatgagaattactgccgaaatccagatgatgatgctcatggaccctggtgctacacgggaaatccactcattccttgggattattgccctatttctcgttgtgaaggtgataccacacctacaatagtcaatttagaccatcccgtaatatcttgtgccaaaacgaaacaattgcgagttgtaaatgggattccaacacgaacaaacataggatggatggttagtttgagatacagaaataaacatatctgcggaggatcattgataaaggagagttgggttcttactgcacgacagtgtttcccttctcgagacttgaaagattatgaagcttggcttggaattcatgatgtccacggaagaggagatgagaaatgcaaacaggttctcaatgtttcccagctggtatatggccctgaaggatcagatctggttttaatgaagcttgccaggcctgctgtcctggatgattttgttagtacgattgatttacctaattatggatgcacaattcctgaaaagaccagttgcagtgtttatggctggggctacactggattgatcaactatgatggcctattacgagtggcacatctctatataatgggaaatgagaaatgcagccagcatcatcgagggaaggtgactctgaatgagtctgaaatatgtgctggggctgaaaagattggatcaggaccatgtgagggggattatggtggcccacttgtttgtgagcaacataaaatgagaatggttcttggtgtcattgttcctggtcgtggatgtgccattccaaatcgtcctggtatttttgtccgagtagcatattatgcaaaatggatacacaaaattattttaacatataaggtaccacagtcatag

SEQ ID NO: 5 - DNA, 3479 bp, synthetic construct
  misc_feature 1..3479: note = HGF-X7-d1
  source 1..3479: mol_type = other DNA
atgtgggtgaccaaactcctgccagccctgctgctgcagcatgtcctcctgcatctcctcctgctccccatcgccatcccctatgcagagggacaaaggaaaagaagaaatacaattcatgaattcaaaaaatcagcaaagactaccctaatcaaaatagatccagcactgaagataaaaaccaaaaaagtgaatactgcagaccaatgtgctaatagatgtactaggaataaaggacttccattcacttgcaaggcttttgtttttgataaagcaagaaaacaatgcctctggttccccttcaatagcatgtcaagtggagtgaaaaaagaatttggccatgaatttgacctctatgaaaacaaagactacattagaaactgcatcattggtaaaggacgcagctacaagggaacagtatctatcactaagagtggcatcaaatgtcagccctggagttccatgataccacacgaacacaggtaagaacagtatgaagaaaagagatgaagcctctgtcttttttacatgttaacagtctcatattagtccttcagaataattctacaatcctaaaataacttagccaacttgctgaattgtattacggcaaggtttatatgaattcatgactgatatttagcaaatgattaattaatatgttaataaaatgtagccaaaacaatatcttaccttaatgcctcaatttgtagatctcggtatttgtggatcctattatgatcttttgtgtaaagtctggcagacaaatgcaatatctaattgttgagtccaatatcacaagcagtacaaaagtataaaaaagacttggccttttctaatgtgttaaaatactttatgctggtaataacactaagagtagggcactagaaattttaagtgaagataatgtgttgcagttactgcactcaatggcttactattataaaccaaaactgggatcactaagctccagtcagtcaaaatgatcaaaattattgaagagaataagcaattctgttctttattaggacacagtagatacagactacaaagtggagtgtgcttaataagaggtagcatttgttaagtgtcaattactctattatcccttggagcttctcaaaataaccatataaggtgtaagatgttaaaggttatggttacactcagtgcacaggtaagctaataggctgagagaagctaaattacttactggggtctcacagtaagaaagtgagctgaagtttcagcccagatttaactggattctgggctctttattcatgttacttcatgaatctgtttctcaattgtgcagaaaaaagggggctatttataagaaaagcaataaacaaacaagtaatgatctcaaataagtaatgcaagaaatagtgagatttcaaaatcagtggcagcgatttctcagttctgtcctaagtggccttgctcaatcacctgctatcttttagtggagctttgaaattatgtttcagacaacttcgattcagttctagaatgtttgactcagcaaattcacaggctcatctttctaacttgatggtgaatatggaaattcagctaaatggatgttaataaaattcaaacgttttaaggacagatggaaatgacagaattttaaggtaaaatatatgaaggaatataagataaaggatttttctaccttcagcaaaaacatacccactaattagtaaaattaataggcgaaaaaaagttgcatgctcttatactgtaatgattatcattttaaaactagctttttgccttcgagctatcggggtaaagacctacaggaaaactactgtcgaaatcctcgaggggaagaagggggaccctggtgtttcacaagcaatccagaggtacgctacgaagtctgtgacattcctcagtgttcagaagttgaatgcatgacctgcaatggggagagttatcgaggtctcatggatcatacagaatcaggcaagatttgtcagcgctgggatcatcagacaccacaccggcacaaattcttgcctgaaagatatcccgacaagggctttgatgataattattgccgcaatcccgatggccagccgaggccatggtgctatactcttgaccctcacacccgctgggagtactgtgcaattaaaacatgcgctgacaatactatgaatgacactgatgttcctttggaaacaactgaatgcatccaaggtcaaggagaaggctacaggggcactgtcaataccatttggaatggaattccatgtcagcgttgggattctcagtatcctcacgagcatgacatgactcctgaaaatttcaagtgcaaggacctacgagaaaattactgccgaaatccagatgggtctgaatcaccctggtgttttaccactgatccaaacatccgagttggctactgctcccaaattccaaactgtgatatgtcacatggacaagattgttatcgtgggaatggcaaaaattatatgggcaacttatcccaaacaagatctggactaacatgttcaatgtgggacaagaacatggaagacttacatcgtcatatcttctgggaaccagatgcaagtaagctgaatgagaattactgccgaaatccagatgatgatgctcatggaccctggtgctacacgggaaatccactcattccttgggattattgccctatttctcgttgtgaaggtgataccacacctacaatagtcaatttagaccatcccgtaatatcttgtgccaaaacgaaacaattgcgagttgtaaatgggattccaacacgaacaaacataggatggatggttagtttgagatacagaaataaacatatctgcggaggatcattgataaaggagagttgggttcttactgcacgacagtgtttcccttctcgagacttgaaagattatgaagcttggcttggaattcatgatgtccacggaagaggagatgagaaatgcaaacaggttctcaatgtttcccagctggtatatggccctgaaggatcagatctggttttaatgaagcttgccaggcctgctgtcctggatgattttgttagtacgattgatttacctaattatggatgcacaattcctgaaaagaccagttgcagtgtttatggctggggctacactggattgatcaactatgatggcctattacgagtggcacatctctatataatgggaaatgagaaatgcagccagcatcatcgagggaaggtgactctgaatgagtctgaaatatgtgctggggctgaaaagattggatcaggaccatgtgagggggattatggtggcccacttgtttgtgagcaacataaaatgagaatggttcttggtgtcattgttcctggtcgtggatgtgccattccaaatcgtcctggtatttttgtccgagtagcatattatgcaaaatggatacacaaaattattttaacatataaggtaccacagtcatag

SEQ ID NO: 6 - DNA, 3279 bp, synthetic construct
  misc_feature 1..3279: note = HGF-X7-d2
  source 1..3279: mol_type = other DNA
atgtgggtgaccaaactcctgccagccctgctgctgcagcatgtcctcctgcatctcctcctgctccccatcgccatcccctatgcagagggacaaaggaaaagaagaaatacaattcatgaattcaaaaaatcagcaaagactaccctaatcaaaatagatccagcactgaagataaaaaccaaaaaagtgaatactgcagaccaatgtgctaatagatgtactaggaataaaggacttccattcacttgcaaggcttttgtttttgataaagcaagaaaacaatgcctctggttccccttcaatagcatgtcaagtggagtgaaaaaagaatttggccatgaatttgacctctatgaaaacaaagactacattagaaactgcatcattggtaaaggacgcagctacaagggaacagtatctatcactaagagtggcatcaaatgtcagccctggagttccatgataccacacgaacacaggtaagaacagtatgaagaaaagagatgaagcctctgtcttttttacatgttaacagtctcatattagtccttcagaataattctacaatcctaaaataacttagccaacttgctgaattgtattacggcaaggtttatatgaattcatgactgatatttagcaaatgattaattaatatgttaataaaatgtagccaaaacaatatcttaccttaatgcctcaatttgtagatctcggtatttgtggatcctttactattataaaccaaaactgggatcactaagctccagtcagtcaaaatgatcaaaattattgaagagaataagcaattctgttctttattaggacacagtagatacagactacaaagtggagtgtgcttaataagaggtagcatttgttaagtgtcaattactctattatcccttggagcttctcaaaataaccatataaggtgtaagatgttaaaggttatggttacactcagtgcacaggtaagctaataggctgagagaagctaaattacttactggggtctcacagtaagaaagtgagctgaagtttcagcccagatttaactggattctgggctctttattcatgttacttcatgaatctgtttctcaattgtgcagaaaaaagggggctatttataagaaaagcaataaacaaacaagtaatgatctcaaataagtaatgcaagaaatagtgagatttcaaaatcagtggcagcgatttctcagttctgtcctaagtggccttgctcaatcacctgctatcttttagtggagctttgaaattatgtttcagacaacttcgattcagttctagaatgtttgactcagcaaattcacaggctcatctttctaacttgatggtgaatatggaaattcagctaaatggatgttaataaaattcaaacgttttaaggacagatggaaatgacagaattttaaggtaaaatatatgaaggaatataagataaaggatttttctaccttcagcaaaaacatacccactaattagtaaaattaataggcgaaaaaaagttgcatgctcttatactgtaatgattatcattttaaaactagctttttgccttcgagctatcggggtaaagacctacaggaaaactactgtcgaaatcctcgaggggaagaagggggaccctggtgtttcacaagcaatccagaggtacgctacgaagtctgtgacattcctcagtgttcagaagttgaatgcatgacctgcaatggggagagttatcgaggtctcatggatcatacagaatcaggcaagatttgtcagcgctgggatcatcagacaccacaccggcacaaattcttgcctgaaagatatcccgacaagggctttgatgataattattgccgcaatcccgatggccagccgaggccatggtgctatactcttgaccctcacacccgctgggagtactgtgcaattaaaacatgcgctgacaatactatgaatgacactgatgttcctttggaaacaactgaatgcatccaaggtcaaggagaaggctacaggggcactgtcaataccatttggaatggaattccatgtcagcgttgggattctcagtatcctcacgagcatgacatgactcctgaaaatttcaagtgcaaggacctacgagaaaattactgccgaaatccagatgggtctgaatcaccctggtgttttaccactgatccaaacatccgagttggctactgctcccaaattccaaactgtgatatgtcacatggacaagattgttatcgtgggaatggcaaaaattatatgggcaacttatcccaaacaagatctggactaacatgttcaatgtgggacaagaacatggaagacttacatcgtcatatcttctgggaaccagatgcaagtaagctgaatgagaattactgccgaaatccagatgatgatgctcatggaccctggtgctacacgggaaatccactcattccttgggattattgccctatttctcgttgtgaaggtgataccacacctacaatagtcaatttagaccatcccgtaatatcttgtgccaaaacgaaacaattgcgagttgtaaatgggattccaacacgaacaaacataggatggatggttagtttgagatacagaaataaacatatctgcggaggatcattgataaaggagagttgggttcttactgcacgacagtgtttcccttctcgagacttgaaagattatgaagcttggcttggaattcatgatgtccacggaagaggagatgagaaatgcaaacaggttctcaatgtttcccagctggtatatggccctgaaggatcagatctggttttaatgaagcttgccaggcctgctgtcctggatgattttgttagtacgattgatttacctaattatggatgcacaattcctgaaaagaccagttgcagtgtttatggctggggctacactggattgatcaactatgatggcctattacgagtggcacatctctatataatgggaaatgagaaatgcagccagcatcatcgagggaaggtgactctgaatgagtctgaaatatgtgctggggctgaaaagattggatcaggaccatgtgagggggattatggtggcccacttgtttgtgagcaacataaaatgagaatggttcttggtgtcattgttcctggtcgtggatgtgccattccaaatcgtcctggtatttttgtccgagtagcatattatgcaaaatggatacacaaaattattttaacatataaggtaccacagtcatag

SEQ ID NO: 7 - DNA, 3079 bp, synthetic construct
  misc_feature 1..3079: note = HGF-X7-d3
  source 1..3079: mol_type = other DNA
atgtgggtgaccaaactcctgccagccctgctgctgcagcatgtcctcctgcatctcctcctgctccccatcgccatcccctatgcagagggacaaaggaaaagaagaaatacaattcatgaattcaaaaaatcagcaaagactaccctaatcaaaatagatccagcactgaagataaaaaccaaaaaagtgaatactgcagaccaatgtgctaatagatgtactaggaataaaggacttccattcacttgcaaggcttttgtttttgataaagcaagaaaacaatgcctctggttccccttcaatagcatgtcaagtggagtgaaaaaagaatttggccatgaatttgacctctatgaaaacaaagactacattagaaactgcatcattggtaaaggacgcagctacaagggaacagtatctatcactaagagtggcatcaaatgtcagccctggagttccatgataccacacgaacacaggtaagaacagtatgaagaaaagagatgaagcctctgtcttttttacatgttaacagtctcatattagtccttcagaataattctacaatcctaaaataacttagccaacttgctgaattgtattacggcaaggtttatatgaattcatgactgatatttagcaaatgattaattaatatgttaataaaatgtagccaaaacaatatcttaccttaatgcctcaatttgtagatctcggtatttgtggatcctaaggtgtaagatgttaaaggttatggttacactcagtgcacaggtaagctaataggctgagagaagctaaattacttactggggtctcacagtaagaaagtgagctgaagtttcagcccagatttaactggattctgggctctttattcatgttacttcatgaatctgtttctcaattgtgcagaaaaaagggggctatttataagaaaagcaataaacaaacaagtaatgatctcaaataagtaatgcaagaaatagtgagatttcaaaatcagtggcagcgatttctcagttctgtcctaagtggccttgctcaatcacctgctatcttttagtggagctttgaaattatgtttcagacaacttcgattcagttctagaatgtttgactcagcaaattcacaggctcatctttctaacttgatggtgaatatggaaattcagctaaatggatgttaataaaattcaaacgttttaaggacagatggaaatgacagaattttaaggtaaaatatatgaaggaatataagataaaggatttttctaccttcagcaaaaacatacccactaattagtaaaattaataggcgaaaaaaagttgcatgctcttatactgtaatgattatcattttaaaactagctttttgccttcgagctatcggggtaaagacctacaggaaaactactgtcgaaatcctcgaggggaagaagggggaccctggtgtttcacaagcaatccagaggtacgctacgaagtctgtgacattcctcagtgttcagaagttgaatgcatgacctgcaatggggagagttatcgaggtctcatggatcatacagaatcaggcaagatttgtcagcgctgggatcatcagacaccacaccggcacaaattcttgcctgaaagatatcccgacaagggctttgatgataattattgccgcaatcccgatggccagccgaggccatggtgctatactcttgaccctcacacccgctgggagtactgtgcaattaaaacatgcgctgacaatactatgaatgacactgatgttcctttggaaacaactgaatgcatccaaggtcaaggagaaggctacaggggcactgtcaataccatttggaatggaattccatgtcagcgttgggattctcagtatcctcacgagcatgacatgactcctgaaaatttcaagtgcaaggacctacgagaaaattactgccgaaatccagatgggtctgaatcaccctggtgttttaccactgatccaaacatccgagttggctactgctcccaaattccaaactgtgatatgtcacatggacaagattgttatcgtgggaatggcaaaaattatatgggcaacttatcccaaacaagatctggactaacatgttcaatgtgggacaagaacatggaagacttacatcgtcatatcttctgggaaccagatgcaagtaagctgaatgagaattactgccgaaatccagatgatgatgctcatggaccctggtgctacacgggaaatccactcattccttgggattattgccctatttctcgttgtgaaggtgataccacacctacaatagtcaatttagaccatcccgtaatatcttgtgccaaaacgaaacaattgcgagttgtaaatgggattccaacacgaacaaacataggatggatggttagtttgagatacagaaataaacatatctgcggaggatcattgataaaggagagttgggttcttactgcacgacagtgtttcccttctcgagacttgaaagattatgaagcttggcttggaattcatgatgtccacggaagaggagatgagaaatgcaaacaggttctcaatgtttcccagctggtatatggccctgaaggatcagatctggttttaatgaagcttgccaggcctgctgtcctggatgattttgttagtacgattgatttacctaattatggatgcacaattcctgaaaagaccagttgcagtgtttatggctggggctacactggattgatcaactatgatggcctattacgagtggcacatctctatataatgggaaatgagaaatgcagccagcatcatcgagggaaggtgactctgaatgagtctgaaatatgtgctggggctgaaaagattggatcaggaccatgtgagggggattatggtggcccacttgtttgtgagcaacataaaatgagaatggttcttggtgtcattgttcctggtcgtggatgtgccattccaaatcgtcctggtatttttgtccgagtagcatattatgcaaaatggatacacaaaattattttaacatataaggtaccacagtcatag

SEQ ID NO: 8 - DNA, 2879 bp, synthetic construct
  misc_feature 1..2879: note = HGF-X7-d4
  source 1..2879: mol_type = other DNA
atgtgggtgaccaaactcctgccagccctgctgctgcagcatgtcctcctgcatctcctcctgctccccatcgccatcccctatgcagagggacaaaggaaaagaagaaatacaattcatgaattcaaaaaatcagcaaagactaccctaatcaaaatagatccagcactgaagataaaaaccaaaaaagtgaatactgcagaccaatgtgctaatagatgtactaggaataaaggacttccattcacttgcaaggcttttgtttttgataaagcaagaaaacaatgcctctggttccccttcaatagcatgtcaagtggagtgaaaaaagaatttggccatgaatttgacctctatgaaaacaaagactacattagaaactgcatcattggtaaaggacgcagctacaagggaacagtatctatcactaagagtggcatcaaatgtcagccctggagttccatgataccacacgaacacaggtaagaacagtatgaagaaaagagatgaagcctctgtcttttttacatgttaacagtctcatattagtccttcagaataattctacaatcctaaaataacttagccaacttgctgaattgtattacggcaaggtttatatgaattcatgactgatatttagcaaatgattaattaatatgttaataaaatgtagccaaaacaatatcttaccttaatgcctcaatttgtagatctcggtatttgtggatccttataagaaaagcaataaacaaacaagtaatgatctcaaataagtaatgcaagaaatagtgagatttcaaaatcagtggcagcgatttctcagttctgtcctaagtggccttgctcaatcacctgctatcttttagtggagctttgaaattatgtttcagacaacttcgattcagttctagaatgtttgactcagcaaattcacaggctcatctttctaacttgatggtgaatatggaaattcagctaaatggatgttaataaaattcaaacgttttaaggacagatggaaatgacagaattttaaggtaaaatatatgaaggaatataagataaaggatttttctaccttcagcaaaaacatacccactaattagtaaaattaataggcgaaaaaaagttgcatgctcttatactgtaatgattatcattttaaaactagctttttgccttcgagctatcggggtaaagacctacaggaaaactactgtcgaaatcctcgaggggaagaagggggaccctggtgtttcacaagcaatccagaggtacgctacgaagtctgtgacattcctcagtgttcagaagttgaatgcatgacctgcaatggggagagttatcgaggtctcatggatcatacagaatcaggcaagatttgtcagcgctgggatcatcagacaccacaccggcacaaattcttgcctgaaagatatcccgacaagggctttgatgataattattgccgcaatcccgatggccagccgaggccatggtgctatactcttgaccctcacacccgctgggagtactgtgcaattaaaacatgcgctgacaatactatgaatgacactgatgttcctttggaaacaactgaatgcatccaaggtcaaggagaaggctacaggggcactgtcaataccatttggaatggaattccatgtcagcgttgggattctcagtatcctcacgagcatgacatgactcctgaaaatttcaagtgcaaggacctacgagaaaattactgccgaaatccagatgggtctgaatcaccctggtgttttaccactgatccaaacatccgagttggctactgctcccaaattccaaactgtgatatgtcacatggacaagattgttatcgtgggaatggcaaaaattatatgggcaacttatcccaaacaagatctggactaacatgttcaatgtgggacaagaacatggaagacttacatcgtcatatcttctgggaaccagatgcaagtaagctgaatgagaattactgccgaaatccagatgatgatgctcatggaccctggtgctacacgggaaatccactcattccttgggattattgccctatttctcgttgtgaaggtgataccacacctacaatagtcaatttagaccatcccgtaatatcttgtgccaaaacgaaacaattgcgagttgtaaatgggattccaacacgaacaaacataggatggatggttagtttgagatacagaaataaacatatctgcggaggatcattgataaaggagagttgggttcttactgcacgacagtgtttcccttctcgagacttgaaagattatgaagcttggcttggaattcatgatgtccacggaagaggagatgagaaatgcaaacaggttctcaatgtttcccagctggtatatggccctgaaggatcagatctggttttaatgaagcttgccaggcctgctgtcctggatgattttgttagtacgattgatttacctaattatggatgcacaattcctgaaaagaccagttgcagtgtttatggctggggctacactggattgatcaactatgatggcctattacgagtggcacatctctatataatgggaaatgagaaatgcagccagcatcatcgagggaaggtgactctgaatgagtctgaaatatgtgctggggctgaaaagattggatcaggaccatgtgagggggattatggtggcccacttgtttgtgagcaacataaaatgagaatggttcttggtgtcattgttcctggtcgtggatgtgccattccaaatcgtcctggtatttttgtccgagtagcatattatgcaaaatggatacacaaaattattttaacatataaggtaccacagtcatag

SEQ ID NO: 9 - DNA, 2879 bp, synthetic construct
  misc_feature 1..2879: note = HGF-X7-d4-codon optimized
  source 1..2879: mol_type = other DNA
atgtgggtcaccaagctgcttcctgctctgctgctccagcacgtgctgctgcacctgctgctgctgcctatcgccatcccctacgccgagggccagagaaagcggagaaacacaatccacgagttcaagaaaagcgccaagacgaccctgatcaagatcgaccccgccctgaagatcaagaccaagaaggtgaacaccgccgaccagtgcgccaaccggtgcaccagaaacaagggcctgcctttcacctgtaaagccttcgtgttcgacaaggccagaaagcagtgtctgtggttccccttcaacagcatgagcagcggcgtgaagaaggaattcggccacgagtttgatctgtacgagaacaaggactacatcagaaattgcatcatcggcaagggcagaagctacaagggtacagtgtccatcactaagagtggcatcaaatgtcagccctggagttccatgataccacacgaacacaggtaagaacagtatgaagaaaagagatgaagcctctgtcttttttacatgttaacagtctcatattagtccttcagaataattctacaatcctaaaataacttagccaacttgctgaattgtattacggcaaggtttatatgaattcatgactgatatttagcaaatgattaattaatatgttaataaaatgtagccaaaacaatatcttaccttaatgcctcaatttgtagatctcggtatttgtggatccttataagaaaagcaataaacaaacaagtaatgatctcaaataagtaatgcaagaaatagtgagatttcaaaatcagtggcagcgatttctcagttctgtcctaagtggccttgctcaatcacctgctatcttttagtggagctttgaaattatgtttcagacaacttcgattcagttctagaatgtttgactcagcaaattcacaggctcatctttctaacttgatggtgaatatggaaattcagctaaatggatgttaataaaattcaaacgttttaaggacagatggaaatgacagaattttaaggtaaaatatatgaaggaatataagataaaggatttttctaccttcagcaaaaacatacccactaattagtaaaattaataggcgaaaaaaagttgcatgctcttatactgtaatgattatcattttaaaactagctttttgccttcgagctatcggggtaaagacttgcaggagaactattgccggaaccccagaggcgaggaaggcggcccctggtgcttcaccagcaaccccgaggtgagatacgaggtgtgcgacatcccccagtgcagcgaggtcgagtgcatgacgtgcaacggcgagagctaccggggcctgatggaccataccgagtctgggaagatctgccagagatgggaccaccagacacctcaccggcacaagttcctgccagaaagatatcctgacaagggcttcgacgataactactgcagaaaccctgacggccaacctagaccttggtgttacacgctggacccccacaccagatgggaatactgtgctattaagacatgtgccgacaataccatgaacgacacagacgtgcctctcgagacaacagaatgcatccagggccagggagaaggatatagaggtacagtgaacaccatctggaacggaattccatgtcagcggtgggacagccaatacccccacgagcacgatatgacccctgagaacttcaagtgtaaagacctgcgggaaaactattgcagaaacccagatggctctgaatctccttggtgcttcacaaccgaccctaatatcagagtgggctactgcagccagatccccaattgcgacatgagccacggacaggactgctacaggggcaatggcaagaactacatgggaaacctgagccagaccagaagcggcctgacctgcagcatgtgggataagaacatggaagatctgcacagacacatcttctgggagcctgatgcttctaagctgaatgagaactactgccggaaccctgatgatgatgcccacggcccctggtgctacactggcaaccccctgatcccatgggactactgtcctatcagcagatgtgaaggcgacaccacacctaccatagttaacctggaccaccccgtgatcagttgcgccaagaccaagcagctgagagtggtgaacggcatccctacaagaaccaacatcggatggatggtgtccctgagatacagaaacaagcacatctgcggcggcagcctgatcaaggaaagctgggtcctcaccgccagacagtgttttcctagccgggacctgaaggactacgaggcctggctgggcatccacgacgtgcacggcagaggcgacgagaagtgcaagcaggtgcttaacgtgtcccaactggtgtacggccccgagggcagtgatctggtgctgatgaaactggccagacccgccgtgctcgacgacttcgtgtctacaatcgacctgcctaactacggctgtaccatccccgagaagaccagctgcagcgtgtacggctggggctatacaggcctcattaactacgacggactgctgagagtggctcacctgtacatcatgggcaacgagaaatgctcccagcaccacagaggcaaggtgaccctgaacgagagcgagatctgtgcaggcgccgagaagatcggcagcggcccttgcgagggcgattacggaggacctctggtctgcgagcagcacaagatgcggatggtcctgggagtgatcgttcctggcagaggatgtgccatccctaacagaccaggaatctttgtgcgggtggcctactacgccaagtggatccacaaaatcatcctgacctacaaggtgccacagtcttga

SEQ ID NO: 10 - DNA, 1070 bp, synthetic construct
  misc_feature 1..1070: note = CMV promoter
  source 1..1070: mol_type = other DNA
cgttacataacttacggtaaatggcccgcctggctgaccgcccaacgacccccgcccattgacgtcaataatgacgtatgttcccatagtaacgccaatagggactttccattgacgtcaatgggtggagtatttacggtaaactgcccacttggcagtacatcaagtgtatcatatgccaagtacgccccctattgacgtcaatgacggtaaatggcccgcctggcattatgcccagtacatgaccttatgggactttcctacttggcagtacatctacgtattagtcatcgctattaccatggtgatgcggttttggcagtacatcaatgggcgtggatagcggtttgactcacggggatttccaagtctccaccccattgacgtcaatgggagtttgttttggcaccaaaatcaacgggactttccaaaatgtcgtaacaactccgccccattgacgcaaatgggcggtaggcgtgtacggtgggaggtctatataagcagagctcgtttagtgaaccgtcagatcgcctggagacgccatccacgctgttttgacctccatagaagacaccgggaccgatccagcctccgcggattcgaatcccggccgggaacggtgcattggaacgcggattccccgtgccaagagtgacgtaagtaccgcctatagagtctataggcccacaaaaaatgctttcttcttttaatatacttttttgtttatcttatttctaatactttccctaatctctttctttcagggcaataatgatacaatgtatcatgcctctttgcaccattctaaagaataacagtgataatttctgggttaaggcaatagcaatatttctgcatataaatatttctgcatataaattgtaactgatgtaagaggtttcatattgctaatagcagctacaatccagctaccattctgcttttattttatggttgggataaggctggattattctgagtccaagctaggcccttttgctaatcatgttcatacctcttatcttcctcccacagctcctgggcaacgtgctggtctgtgtgctggccca

SEQ ID NO: 11 - DNA, 1160 bp, synthetic construct
  misc_feature 1..1160: note = CMV promoter
  source 1..1160: mol_type = other DNA
ctagttattaatagtaatcaattacggggtcattagttcatagcccatatatggagttccgcgttacataacttacggtaaatggcccgcctggctgaccgcccaacgacccccgcccattgacgtcaataatgacgtatgttcccatagtaacgccaatagggactttccattgacgtcaatgggtggagtatttacggtaaactgcccacttggcagtacatcaagtgtatcatatgccaagtacgccccctattgacgtcaatgacggtaaatggcccgcctggcattatgcccagtacatgaccttatgggactttcctacttggcagtacatctacgtattagtcatcgctattaccatggtgatgcggttttggcagtacatcaatgggcgtggatagcggtttgactcacggggatttccaagtctccaccccattgacgtcaatgggagtttgttttggcaccaaaatcaacgggactttccaaaatgtcgtaacaactccgccccattgacgcaaatgggcggtaggcgtgtacggtgggaggtctatataagcagagctcgtttagtgaaccgtcagatcgcctggagacgccatccacgctgttttgacctccatagaagacaccgggaccgatccagcctccgcggattcgaatcccggccgggaacggtgcattggaacgcggattccccgtgccaagagtgacgtaagtaccgcctatagagtctataggcccacaaaaaatgctttcttcttttaatatacttttttgtttatcttatttctaatactttccctaatctctttctttcagggcaataatgatacaatgtatcatgcctctttgcaccattctaaagaataacagtgataatttctgggttaaggcaatagcaatatttctgcatataaatatttctgcatataaattgtaactgatgtaagaggtttcatattgctaatagcagctacaatccagctaccattctgcttttattttatggttgggataaggctggattattctgagtccaagctaggcccttttgctaatcatgttcatacctcttatcttcctcccacagctcctgggcaacgtgctggtctgtgtgctggcccatcactttggcaaagaattgggattcgaac

SEQ ID NO: 12 - DNA, 784 bp, synthetic construct
  misc_feature 1..784: note = EF-1alpha promoter
  source 1..784: mol_type = other DNA
ggcaattgaaccggtgcctagagaaggtggcgcggggtaaactgggaaagtgatgtcgtgtactggctccgcctttttcccgagggtgggggagaaccgtatataagtgcagtagtcgccgtgaacgttctttttcgcaacgggtttgccgccagaacacaggtaagtgccgtgtgtggttcccgcgggcggcgacggggcccgtgcgtcccagcgcacatgttcggcgaggcggggcctgcgagcgcggccaccgagaatcggacgggggtagtctcaagctggccggcctgctctggtgcctggcctcgcgccgccgtgtatcgccccgccctgggcggcaaggctggcccggtcggcaccagttgcgtgagcggaaagatggccgcttcccggccctgctgcagggagctcaaaatggaggacgcggcgctcgggagagcgggcgggtgagtcacccacacaaaggaaaagggcctttccgtcctcagccgtcgcttcatgtgactccacggagtaccgggcgccgtccaggcacctcgattagttctcgagcttttggagtacgtcgtctttaggttggggggaggggttttatgcgatggagtttccccacactgagtgggtggagactgaagttaggccagcttggcacttgatgtaattctccttggaatttgccctttttgagtttggatcttggttcattctcaagcctcagacagtggttcaaagtttgttccttccatttcaggtgtcgtgaaaactacccctaaaagccaaa

SEQ ID NO: 13 - DNA, 477 bp, synthetic construct
  misc_feature 1..477: note = hGH pA
  source 1..477: mol_type = other DNA
gggtggcatccctgtgacccctccccagtgcctctcctggccctggaagttgccactccagtgcccaccagccttgtcctaataaaattaagttgcatcattttgtctgactaggtgtccttctataatattatggggtggaggggggtggtatggagcaaggggcaagttgggaagacaacctgtagggcctgcggggtctattgggaaccaagctggagtgcagtggcacaatcttggctcactgcaatctccgcctcctgggttcaagcgattctcctgcctcagcctcccgagttgttgggattccaggcatgcatgaccaggctcagctaatttttgtttttttggtagagacggggtttcaccatattggccaggctggtctccaactcctaatctcaggtgatctacccaccttggcctcccaaattgctgggattacaggcgtgaaccactgctcccttccctgtcctt

SEQ ID NO: 14 - DNA, 542 bp, synthetic construct
  misc_feature 1..542: note = hGH pA
  source 1..542: mol_type = other DNA
ctgcagaagcttgcctcgagcagcgctgctcgagagatctacgggtggcatccctgtgacccctccccagtgcctctcctggccctggaagttgccactccagtgcccaccagccttgtcctaataaaattaagttgcatcattttgtctgactaggtgtccttctataatattatggggtggaggggggtggtatggagcaaggggcaagttgggaagacaacctgtagggcctgcggggtctattgggaaccaagctggagtgcagtggcacaatcttggctcactgcaatctccgcctcctgggttcaagcgattctcctgcctcagcctcccgagttgttgggattccaggcatgcatgaccaggctcagctaatttttgtttttttggtagagacggggtttcaccatattggccaggctggtctccaactcctaatctcaggtgatctacccaccttggcctcccaaattgctgggattacaggcgtgaaccactgctcccttccctgtccttctgattttgtaggtaaccacgtg

SEQ ID NO: 15 - DNA, 208 bp, synthetic construct
  misc_feature 1..208: note = bGH pA
  source 1..208: mol_type = other DNA
ctgtgccttctagttgccagccatctgttgtttgcccctcccccgtgccttccttgaccctggaaggtgccactcccactgtcctttcctaataaaatgaggaaattgcatcgcattgtctgagtaggtgtcattctattctggggggtggggtggggcaggacagcaagggggaggattgggaagacaatagcaggcatgctgggga

SEQ ID NO: 16 - DNA, 317 bp, synthetic construct
  misc_feature 1..317: note = bGH pA
  source 1..317: mol_type = other DNA
ctgcagaagcttgcctcgagcagcgctcgagagagatctctcgagtctagagggcccgtttaaacccgctgatcagcctcgactgtgccttctagttgccagccatctgttgtttgcccctcccccgtgccttccttgaccctggaaggtgccactcccactgtcctttcctaataaaatgaggaaattgcatcgcattgtctgagtaggtgtcattctattctggggggtggggtggggcaggacagcaagggggaggattgggaagacaatagcaggcatgctggggagtcgctgattttgtaggtaaccacgtg

SEQ ID NO: 17 - DNA, 68 bp, synthetic construct
  misc_feature 1..68: note = SV40 pA
  source 1..68: mol_type = other DNA
aacttgtttattgcagcttataatggttacaaataaagcaatagcatcacaaatttcacaaataaagc

SEQ ID NO: 18 - DNA, 185 bp, synthetic construct
  misc_feature 1..185: note = SV40 pA
  source 1..185: mol_type = other DNA
ctgcagaagcttgcctcgagcagcgctgctcgagagatctaacttgtttattgcagcttataatggttacaaataaagcaatagcatcacaaatttcacaaataaagcatttttttcactgcattctagttgtggtttgtccaaactcatcaatgtatcttactgattttgtaggtaaccacgtg

SEQ ID NO: 19 - DNA, 2730 bp, synthetic construct
  misc_feature 1..2730: note = HGF-X8
  source 1..2730: mol_type = other DNA
atgtgggtgaccaaactcctgccagccctgctgctgcagcatgtcctcctgcatctcctcctgctccccatcgccatcccctatgcagagggacaaaggaaaagaagaaatacaattcatgaattcaaaaaatcagcaaagactaccctaatcaaaatagatccagcactgaagataaaaaccaaaaaagtgaatactgcagaccaatgtgctaatagatgtactaggaataaaggacttccattcacttgcaaggcttttgtttttgataaagcaagaaaacaatgcctctggttccccttcaatagcatgtcaagtggagtgaaaaaagaatttggccatgaatttgacctctatgaaaacaaagactacattagaaactgcatcattggtaaaggacgcagctacaagggaacagtatctatcactaagagtggcatcaaatgtcagccctggagttccatgataccacacgaacacaggtaagaacagtatgaagaaaagagatgaagcctctgtcttttttacatgttaacagtctcatattagtccttcagaataattctacaatcctaaaataacttagccaacttgctgaattgtattacggcaaggtttatatgaattcatgactgatatttagcaaatgattaattaatatgttaataaaatgtagccaaaacaatatcttaccttaatgcctcaatttgtagatctcggtatttgtggatccttatgtttcagacaacttcgattcagttctagaatgtttgactcagcaaattcacaggctcatctttctaacttgatggtgaatatggaaattcagctaaatggatgttaataaaattcaaacgttttaaggacagatggaaatgacagaattttaaggtaaaatatatgaaggaatataagataaaggatttttctaccttcagcaaaaacatacccactaattagtaaaattaataggcgaaaaaaagttgcatgctcttatactgtaatgattatcattttaaaactagctttttgccttcgagctatcggggtaaagacctacaggaaaactactgtcgaaatcctcgaggggaagaagggggaccctggtgtttcacaagcaatccagaggtacgctacgaagtctgtgacattcctcagtgttcagaagttgaatgcatgacctgcaatggggagagttatcgaggtctcatggatcatacagaatcaggcaagatttgtcagcgctgggatcatcagacaccacaccggcacaaattcttgcctgaaagatatcccgacaagggctttgatgataattattgccgcaatcccgatggccagccgaggccatggtgctatactcttgaccctcacacccgctgggagtactgtgcaattaaaacatgcgctgacaatactatgaatgacactgatgttcctttggaaacaactgaatgcatccaaggtcaaggagaaggctacaggggcactgtcaataccatttggaatggaattccatgtcagcgttgggattctcagtatcctcacgagcatgacatgactcctgaaaatttcaagtgcaaggacctacgagaaaattactgccgaaatccagatgggtctgaatcaccctggtgttttaccactgatccaaacatccgagttggctactgctcccaaattccaaactgtgatatgtcacatggacaagattgttatcgtgggaatggcaaaaattatatgggcaacttatcccaaacaagatctggactaacatgttcaatgtgggacaagaacatggaagacttacatcgtcatatcttctgggaaccagatgcaagtaagctgaatgagaattactgccgaaatccagatgatgatgctcatggaccctggtgctacacgggaaatccactcattccttgggattattgccctatttctcgttgtgaaggtgataccacacctacaatagtcaatttagaccatcccgtaatatcttgtgccaaaacgaaacaattgcgagttgtaaatgggattccaacacgaacaaacataggatggatggttagtttgagatacagaaataaacatatctgcggaggatcattgataaaggagagttgggttcttactgcacgacagtgtttcccttctcgagacttgaaagattatgaagcttggcttggaattcatgatgtccacggaagaggagatgagaaatgcaaacaggttctcaatgtttcccagctggtatatggccctgaaggatcagatctggttttaatgaagcttgccaggcctgctgtcctggatgattttgttagtacgattgatttacctaattatggatgcacaattcctgaaaagaccagttgcagtgtttatggctggggctacactggattgatcaactatgatggcctattacgagtggcacatctctatataatgggaaatgagaaatgcagccagcatcatcgagggaaggtgactctgaatgagtctgaaatatgtgctggggctgaaaagattggatcaggaccatgtgagggggattatggtggcccacttgtttgtgagcaacataaaatgagaatggttcttggtgtcattgttcctggtcgtggatgtgccattccaaatcgtcctggtatttttgtccgagtagcatattatgcaaaatggatacacaaaattattttaacatataaggtaccacagtcatag

SEQ ID NO: 20 - DNA, 2910 bp, synthetic construct
  misc_feature 1..2910: note = backbone
  source 1..2910: mol_type = other DNA
cggaccgagcggccgcaggaacccctagtgatggagttggccactccctctctgcgcgctcgctcgctcactgaggccgggcgaccaaaggtcgcccgacgcccgggctttgcccgggcggcctcagtgagcgagcgagcgcgcagctgcctgcaggggcgcctgatgcggtattttctccttacgcatctgtgcggtatttcacaccgcatacgtcaaagcaaccatagtacgcgccctgtagcggcgcattaagcgcggcgggtgtggtggttacgcgcagcgtgaccgctacacttgccagcgccttagcgcccgctcctttcgctttcttcccttcctttctcgccacgttcgccggctttccccgtcaagctctaaatcgggggctccctttagggttccgatttagtgctttacggcacctcgaccccaaaaaacttgatttgggtgatggttcacgtagtgggccatcgccctgatagacggtttttcgccctttgacgttggagtccacgttctttaatagtggactcttgttccaaactggaacaacactcaactctatctcgggctattcttttgatttataagggattttgccgatttcggtctattggttaaaaaatgagctgatttaacaaaaatttaacgcgaattttaacaaaatattaacgtttacaattttatggtgcactctcagtacaatctgctctgatgccgcatagttaagccagccccgacacccgccaacacccgctgacgcgccctgacgggcttgtctgctcccggcatccgcttacagacaagctgtgaccgtctccgggagctgcatgtgtcagaggttttcaccgtcatcaccgaaacgcgcgagacgaaagggcctcgtgatacgcctatttttataggttaatgtcatgataataatggtttcttagacgtcaggtggcacttttcggggaaatgtgcgcggaacccctatttgtttatttttctaaatacattcaaatatgtatccgctcatgagacaataaccctgataaatgcttcaataatattgaaaaaggaagagtatgagtattcaacatttccgtgtcgcccttattcccttttttgcggcattttgccttcctgtttttgctcacccagaaacgctggtgaaagtaaaagatgctgaagatcagttgggtgcacgagtgggttacatcgaactggatctcaacagcggtaagatccttgagagttttcgccccgaagaacgttttccaatgatgagcacttttaaagttctgctatgtggcgcggtattatcccgtattgacgccgggcaagagcaactcggtcgccgcatacactattctcagaatgacttggttgagtactcaccagtcacagaaaagcatcttacggatggcatgacagtaagagaattatgcagtgctgccataaccatgagtgataacactgcggccaacttacttctgacaacgatcggaggaccgaaggagctaaccgcttttttgcacaacatgggggatcatgtaactcgccttgatcgttgggaaccggagctgaatgaagccataccaaacgacgagcgtgacaccacgatgcctgtagcaatggcaacaacgttgcgcaaactattaactggcgaactacttactctagcttcccggcaacaattaatagactggatggaggcggataaagttgcaggaccacttctgcgctcggcccttccggctggctggtttattgctgataaatctggagccggtgagcgtgggtctcgcggtatcattgcagcactggggccagatggtaagccctcccgtatcgtagttatctacacgacggggagtcaggcaactatggatgaacgaaatagacagatcgctgagataggtgcctcactgattaagcattggtaactgtcagaccaagtttactcatatatactttagattgatttaaaacttcatttttaatttaaaaggatctaggtgaagatcctttttgataatctcatgaccaaaatcccttaacgtgagttttcgttccactgagcgtcagaccccgtagaaaagatcaaaggatcttcttgagatcctttttttctgcgcgtaatctgctgcttgcaaacaaaaaaaccaccgctaccagcggtggtttgtttgccggatcaagagctaccaactctttttccgaaggtaactggcttcagcagagcgcagataccaaatactgttcttctagtgtagccgtagttaggccaccacttcaagaactctgtagcaccgcctacatacctcgctctgctaatcctgttaccagtggctgctgccagtggcgataagtcgtgtcttaccgggttggactcaagacgatagttaccggataaggcgcagcggtcgggctgaacggggggttcgtgcacacagcccagcttggagcgaacgacctacaccgaactgagatacctacagcgtgagctatgagaaagcgccacgcttcccgaagggagaaaggcggacaggtatccggtaagcggcagggtcggaacaggagagcgcacgagggagcttccagggggaaacgcctggtatctttatagtcctgtcgggtttcgccacctctgacttgagcgtcgatttttgtgatgctcgtcaggggggcggagcctatggaaaaacgccagcaacgcggcctttttacggttcctggccttttgctggccttttgctcacatgtcctgcaggcagctgcgcgctcgctcgctcactgaggccgcccgggcgtcgggcgacctttggtcgcccggcctcagtgagcgagcgagcgcgcagagagggagtggccaactccatcactaggggttcctgcggccgcacgcgtatcgatgtcgac